European Patent Application EP 4 571 315 A1, published June 18, 2025. Title: DIAGNOSTIC USE OF HIGHLY TOXIC AMYLOID OLIGOMER. Applicant: Shen Zhen Wisdom Biopharm Co., Ltd. The sequence listing filed with the application follows.

SEQUENCE LISTING (29 sequences)

SEQ ID NO: 1 - DNA, 20 bp, synthetic construct
  misc_feature 1..20: note = mTNF- Forw
  source 1..20: mol_type = other DNA
gattatggctcagggtccaa

SEQ ID NO: 2 - DNA, 20 bp, synthetic construct
  misc_feature 1..20: note = mTNF- rever
  source 1..20: mol_type = other DNA
gctccagtgaattcggaaag

SEQ ID NO: 3 - DNA, 20 bp, synthetic construct
  misc_feature 1..20: note = mIL-1 forw
  source 1..20: mol_type = other DNA
cccaagcaatacccaaagaa

SEQ ID NO: 4 - DNA, 20 bp, synthetic construct
  misc_feature 1..20: note = mIL-1 rever
  source 1..20: mol_type = other DNA
gcttgtgctctgcttgtgag

SEQ ID NO: 5 - DNA, 20 bp, synthetic construct
  misc_feature 1..20: note = mIL-6 forw
  source 1..20: mol_type = other DNA
ccggagaggagacttcacag

SEQ ID NO: 6 - DNA, 20 bp, synthetic construct
  misc_feature 1..20: note = mIL-6 rever
  source 1..20: mol_type = other DNA
ttgccattgcacaactcttt

SEQ ID NO: 7 - DNA, 20 bp, synthetic construct
  misc_feature 1..20: note = GAPDH forw
  source 1..20: mol_type = other DNA
tgaatacggctacagcaaca

SEQ ID NO: 8 - DNA, 20 bp, synthetic construct
  misc_feature 1..20: note = GAPDH rever
  source 1..20: mol_type = other DNA
aggcccctcctgttattatg

SEQ ID NO: 9 - DNA, 20 bp, synthetic construct
  misc_feature 1..20: note = miNos forw
  source 1..20: mol_type = other DNA
cacctggaacagcactctct

SEQ ID NO: 10 - DNA, 20 bp, synthetic construct
  misc_feature 1..20: note = miNos rever
  source 1..20: mol_type = other DNA
ctttgtgcgaagtgtcagtg

SEQ ID NO: 11 - DNA, 21 bp, synthetic construct
  misc_feature 1..21: note = mGpc4 forw
  source 1..21: mol_type = other DNA
ctggagggtcctttcaacatt

SEQ ID NO: 12 - DNA, 21 bp, synthetic construct
  misc_feature 1..21: note = mGpc4 rever
  source 1..21: mol_type = other DNA
gacatcagtaaccagtcggtc

SEQ ID NO: 13 - DNA, 21 bp, synthetic construct
  misc_feature 1..21: note = mGpc6 forw
  source 1..21: mol_type = other DNA
tagtcctgtattggcagccac

SEQ ID NO: 14 - DNA, 22 bp, synthetic construct
  misc_feature 1..22: note = mGpc6 rever
  source 1..22: mol_type = other DNA
ggctaatgtctatagcagggaa

SEQ ID NO: 15 - DNA, 22 bp, synthetic construct
  misc_feature 1..22: note = mTSP1 forw
  source 1..22: mol_type = other DNA
ggtagctggaaatgtggtgcgt

SEQ ID NO: 16 - DNA, 22 bp, synthetic construct
  misc_feature 1..22: note = mTSP1
  source 1..22: mol_type = other DNA
gcaccgatgttctccgttgtga

SEQ ID NO: 17 - protein, 5 aa, synthetic construct
  REGION 1..5: note = 3F VH-CDR1
SYAMS

SEQ ID NO: 18 - protein, 17 aa, synthetic construct
  REGION 1..17: note = 3F VH-CDR2
GISNLGLTTGYADSVKG

SEQ ID NO: 19 - protein, 7 aa, synthetic construct
  REGION 1..7: note = 3F VH-CDR3
TTSRFDY

SEQ ID NO: 20 - protein, 11 aa, synthetic construct
  REGION 1..11: note = 3F VL-CDR1
RASQSISSYLN

SEQ ID NO: 21 - protein, 7 aa, synthetic construct
  REGION 1..7: note = 3F VL-CDR2
KASYLQS

SEQ ID NO: 22 - protein, 9 aa, synthetic construct
  REGION 1..9: note = 3F VL-CDR3
QNSAVRPVT

SEQ ID NO: 23 - protein, 242 aa, synthetic construct
  REGION 1..242: note = 3F
MAEVQLLESGGGLVQPGGSLRLSCAASGFTFSSYAMSWVRQAPGKGLEWVSGISNLGLTTGYADSVKGRFTISRDNSKNTLYLQMNSLRAEDTAVYYCAKTTSRFDYWGQGTLVTVSSGGGGSGGGGSGGGGSTDIQMTQSPSSLSASVGDRVTITCRASQSISSYLNWYQQKPGKAPKLLIYKASYLQSGVPSRFSGSGSGTDFTLTISSLQPEDFATYYCQNSAVRPVTFGQGTKVEIKR

SEQ ID NO: 24 - protein, 242 aa, synthetic construct
MAEVQLLESGGGLVQPGGSLRLSCAASGFTFSSYAMSWVRQAPGKGLEWVSGISNLGLTTGYADSVKGRFTISRDNSKNTLYLQMNSLRAEDTAVYYCARTTSRFDYWGQGTLVTVSSGGGGSGGGGSGGGGSTDIQMTQSPSSLSASVGDRVTITCRASQSISSYLNWYQQKPGKAPKLLIYKASYLQSGVPSRFSGSGSGTDFTLTISSLQPEDFATYYCQNSAVRPVTFGQGTKVEIKR

SEQ ID NO: 25 - protein, 8 aa, synthetic construct
GFTFSSYA

SEQ ID NO: 26 - protein, 8 aa, synthetic construct
ISNLGLTT

SEQ ID NO: 27 - protein, 9 aa, synthetic construct
AKTTSRFDY

SEQ ID NO: 28 - protein, 6 aa, synthetic construct
QSISSY

SEQ ID NO: 29 - protein, 9 aa, synthetic construct
QNSAVRPVT